European Patent Specification EP 3 949 990 B1, published July 8, 2026. Title: A pharmaceutical combination for treating tumor. Applicant: Chiome Bioscience Inc. The sequence listing filed with the application follows.

SEQUENCE LISTING (46 sequences)

SEQ ID NO: 1 - DNA, 1532 bp, Homo sapiens
  CDS (154)..(1305)
gagagcgcagcgcgcagcccggtgcagccctggctttcccctcgctgcgcgcccgcgccccctttcgcgtccgcaaccagaagcccagtgcggcgccaggagccggacccgcgcccgcaccgctcccgggaccgcgaccccggccgcccagagatgaccgcgaccgaagccctcctgcgcgtcctcttgctcctgctggctttcggccacagcacctatggggctgaatgcttcccggcctgcaacccccaaaatggattctgcgaggatgacaatgtttgcaggtgccagcctggctggcagggtcccctttgtgaccagtgcgtgacctctcccggctgccttcacggactctgtggagaacccgggcagtgcatttgcaccgacggctgggacggggagctctgtgatagagatgttcgggcctgctcctcggccccctgtgccaacaacgggacctgcgtgagcctggacgatggcctctatgaatgctcctgtgcccccgggtactcgggaaaggactgccagaaaaaggacgggccctgtgtgatcaacggctccccctgccagcacggaggcacctgcgtggatgatgagggccgggcctcccatgcctcctgcctgtgcccccctggcttctcaggcaatttctgcgagatcgtggccaacagctgcacccccaacccatgcgagaacgacggcgtctgcactgacattgggggcgacttccgctgccggtgcccagccggcttcatcgacaagacctgcagccgcccggtgaccaactgcgccagcagcccgtgccagaacgggggcacctgcctgcagcacacccaggtgagctacgagtgtctgtgcaagcccgagttcacaggtctcacctgtgtcaagaagcgcgcgctgagcccccagcaggtcacccgtctgcccagcggctatgggctggcctaccgcctgacccctggggtgcacgagctgccggtgcagcagccggagcaccgcatcctgaaggtgtccatgaaagagctcaacaagaaaacccctctcctcaccgagggccaggccatctgcttcaccatcctgggcgtgctcaccagcctggtggtgctgggcactgtgggtatcgtcttcctcaacaagtgcgagacctgggtgtccaacctgcgctacaaccacatgctgcggaagaagaagaacctgctgcttcagtacaacagcggggaggacctggccgtcaacatcatcttccccgagaagatcgacatgaccaccttcagcaaggaggccggcgacgaggagatctaagcagcgttcccacagccccctctagattcttggagttccgcagagcttactatacgcggtctgtcctaatctttgtggtgttcgctatctcttgtgtcaaatctggtgaacgctacgcttacatatattgtctttgtgctgctgtgtgacaaacgcaatgcaaaaacaatcctctttctctctcttaatgcatgatacagaataataataagaatttcatctttaaa

SEQ ID NO: 2 - protein, 383 aa, Homo sapiens
MTATEALLRVLLLLLAFGHSTYGAECFPACNPQNGFCEDDNVCRCQPGWQGPLCDQCVTSPGCLHGLCGEPGQCICTDGWDGELCDRDVRACSSAPCANNGTCVSLDDGLYECSCAPGYSGKDCQKKDGPCVINGSPCQHGGTCVDDEGRASHASCLCPPGFSGNFCEIVANSCTPNPCENDGVCTDIGGDFRCRCPAGFIDKTCSRPVTNCASSPCQNGGTCLQHTQVSYECLCKPEFTGLTCVKKRALSPQQVTRLPSGYGLAYRLTPGVHELPVQQPEHRILKVSMKELNKKTPLLTEGQAICFTILGVLTSLVVLGTVGIVFLNKCETWVSNLRYNHMLRKKKNLLLQYNSGEDLAVNIIFPEKIDMTTFSKEAGDEEI

SEQ ID NO: 3 - protein, 5 aa, Mus musculus
DTYIH

SEQ ID NO: 4 - protein, 17 aa, Mus musculus
RIDPPNGNLKYDPKFQG

SEQ ID NO: 5 - protein, 8 aa, Mus musculus
SDGYSFAY

SEQ ID NO: 6 - protein, 16 aa, Mus musculus
RSSKSLLHSNGNTYLY

SEQ ID NO: 7 - protein, 7 aa, Mus musculus
RMSNLAS

SEQ ID NO: 8 - protein, 9 aa, Mus musculus
MQHVEYPFT

SEQ ID NO: 9 - protein, 5 aa, Mus musculus
DYAMH

SEQ ID NO: 10 - protein, 17 aa, Mus musculus
VISTYYGNTNYNQKFKG

SEQ ID NO: 11 - protein, 12 aa, Mus musculus
GGLREYYYAMDY

SEQ ID NO: 12 - protein, 17 aa, Mus musculus
KSSQSLLNSSNQKNYLA

SEQ ID NO: 13 - protein, 7 aa, Mus musculus
FASTRES

SEQ ID NO: 14 - protein, 9 aa, Mus musculus
QQHYSTPPT

SEQ ID NO: 15 - DNA, 354 bp, Mus musculus
  CDS (1)..(354)
gaggttcagctgcagcagtctggggcagagcttgtgaagccaggggcctcagtcaagttgtcctgcacagcttctggcttcaacattagagacacctatatacactgggtgaagcagaggcctgagcagggcctggagtggattggaaggattgatcctccgaatggtaatcttaaatatgacccgaagttccagggcaaggccactataacagcagacacatcctccaacacagcctacctgcagttcagcagcctgacatctgaggacactgccgtctattactgtgcaaggtctgatggttactcctttgcttactggggccaagggactctggtcactgtctctgcagcc

SEQ ID NO: 16 - protein, 118 aa, Mus musculus
EVQLQQSGAELVKPGASVKLSCTASGFNIRDTYIHWVKQRPEQGLEWIGRIDPPNGNLKYDPKFQGKATITADTSSNTAYLQFSSLTSEDTAVYYCARSDGYSFAYWGQGTLVTVSAA

SEQ ID NO: 17 - DNA, 336 bp, Mus musculus
  CDS (1)..(336)
gatattgtgatgactcaggctgcaccctctgtacctgtcactcctggagagtcagtatccatctcctgcaggtctagtaagagtctcctgcatagtaatggcaacacttacttgtattggttcctgcagaggccaggccagtctcctcagctcctgatatatcggatgtccaaccttgcctcaggagtcccagacaggttcagtggcagtgggtcaggaactgctttcacactgagaatcagtagagtggaggctgaggatgtgggtgtttattactgtatgcaacatgtagaatatccattcacgttcggctcggggacaaagttggaaataaaa

SEQ ID NO: 18 - protein, 112 aa, Mus musculus
DIVMTQAAPSVPVTPGESVSISCRSSKSLLHSNGNTYLYWFLQRPGQSPQLLIYRMSNLASGVPDRFSGSGSGTAFTLRISRVEAEDVGVYYCMQHVEYPFTFGSGTKLEIK

SEQ ID NO: 19 - DNA, 363 bp, Mus musculus
  CDS (1)..(363)
caggtccagctgcagcagtctgggcctgagctggtgaggcctggggtctcagtgaagatttcctgcaagggttccggctacacattcactgattatgctatgcactgggtgaagcagagtcatgcaaagagtctagagtggattggagttattagtacttactatggtaatacaaactacaaccagaagtttaagggcaaggccacaatgactgtagacaaatcctccagcacagcctatatggaacttgccagattgacatctgaggattctgccatctattactgtgcaagaggaggattacgagagtattactatgctatggactactggggtcaaggaacctcagtcaccgtctcctca

SEQ ID NO: 20 - protein, 121 aa, Mus musculus
QVQLQQSGPELVRPGVSVKISCKGSGYTFTDYAMHWVKQSHAKSLEWIGVISTYYGNTNYNQKFKGKATMTVDKSSSTAYMELARLTSEDSAIYYCARGGLREYYYAMDYWGQGTSVTVSS

SEQ ID NO: 21 - DNA, 339 bp, Mus musculus
  CDS (1)..(339)
gacattgtgatgacacagtctccatcctccctggctatgtcagtaggacagaaggtcactatgagctgcaagtccagtcagagccttttaaatagtagcaatcaaaagaactatttggcctggtaccagcagaaaccaggacagtctcctaaacttctggtatactttgcatccactagggaatctggggtccctgatcgcttcataggcagtggatctgggacagatttcactcttaccatcagcagtgtgcaggctgaagacctggcagattacttctgtcagcaacattatagcactcctcccacgttcggtgctgggaccaagctggagctgaaa

SEQ ID NO: 22 - protein, 113 aa, Mus musculus
DIVMTQSPSSLAMSVGQKVTMSCKSSQSLLNSSNQKNYLAWYQQKPGQSPKLLVYFASTRESGVPDRFIGSGSGTDFTLTISSVQAEDLADYFCQQHYSTPPTFGAGTKLELK

SEQ ID NO: 23 - DNA, 351 bp, Artificial
  Recombinant DNA
  CDS (1)..(351)
caggttcagctggtgcagtctggggcagaggtgaagaagccagggtcctcagtcaaggtctcctgcaaggcttctggcttcaacattagagacacctatatacactgggtgcggcaggcccctggacagggcctggagtggattggaaggattgatcctccgaatggtaatcttaaatatgacccgaagttccagggcaaggccactataacagcagacacatccacgagcacagcctacatggagttcagcagcctgagatctgaggacactgccgtctattactgtgcaaggtctgatggttactcctttgcttactggggccaagggactctggtcactgtctcttca

SEQ ID NO: 24 - protein, 117 aa, Artificial
  Synthetic Construct (Recombinant Protein)
QVQLVQSGAEVKKPGSSVKVSCKASGFNIRDTYIHWVRQAPGQGLEWIGRIDPPNGNLKYDPKFQGKATITADTSTSTAYMEFSSLRSEDTAVYYCARSDGYSFAYWGQGTLVTVSS

SEQ ID NO: 25 - DNA, 351 bp, Artificial
  Recombinant DNA
  CDS (1)..(351)
caggttcagctggtgcagtctggggcagaggtgaagaagccagggtcctcagtcaaggtctcctgcaaggcttctggcttcaacattagagacacctatatacactgggtgcggcaggcccctggacagggcctggagtggattggaaggattgatcctccgaatggtaatcttaaatatgacccgaagttccagggcaaggccactataacagcagacacatccacgagcacagcctacatggagctgagcagcctgagatctgaggacactgccgtctattactgtgcaaggtctgatggttactcctttgcttactggggccaaggaactctggtcactgtctcttca

SEQ ID NO: 26 - protein, 117 aa, Artificial
  Synthetic Construct (Recombinant Protein)
QVQLVQSGAEVKKPGSSVKVSCKASGFNIRDTYIHWVRQAPGQGLEWIGRIDPPNGNLKYDPKFQGKATITADTSTSTAYMELSSLRSEDTAVYYCARSDGYSFAYWGQGTLVTVSS

SEQ ID NO: 27 - DNA, 336 bp, Artificial
  Recombinant DNA
  CDS (1)..(336)
gatattgtgatgactcagtctccactctctctgcctgtcactcctggagagccggcctccatctcctgcaggtctagcaagagtctcctgcatagtaatggcaacacttacttgtattggttcctgcagaagccaggccagtctcctcagctcctgatatatcggatgtccaaccttgcctcaggagtcccagacaggttcagtggcagtgggtcaggaactgctttcacactgaaaatcagtagagtggaggctgaggatgtgggtgtttattactgtatgcaacatgtagaatatccattcacgttcggccaagggacaaaggtggaaatcaaa

SEQ ID NO: 28 - protein, 112 aa, Artificial
  Synthetic Construct (Recombinant Protein)
DIVMTQSPLSLPVTPGEPASISCRSSKSLLHSNGNTYLYWFLQKPGQSPQLLIYRMSNLASGVPDRFSGSGSGTAFTLKISRVEAEDVGVYYCMQHVEYPFTFGQGTKVEIK

SEQ ID NO: 29 - DNA, 363 bp, Artificial
  Recombinant DNA
  CDS (1)..(363)
caagtccagctggtgcagtctggggctgaagtgaagaagcctggggcctcagtgaaagtctcctgcaaggcttccggctacacattcactgattatgctatgcactgggtgcgacaggcccctggacaaggcctggagtggattggagttattagtacttactatggtaatacaaactacaaccagaagtttaagggcaaggccacaatgactgtcgacacatccaccagcacagcctatatggaacttaggagcttgagatctgacgatactgccgtgtattactgtgcaagaggaggattgcgagagtattactatgctatggactactggggtcaaggaaccatggtcaccgtctcctca

SEQ ID NO: 30 - protein, 121 aa, Artificial
  Synthetic Construct (Recombinant Protein)
QVQLVQSGAEVKKPGASVKVSCKASGYTFTDYAMHWVRQAPGQGLEWIGVISTYYGNTNYNQKFKGKATMTVDTSTSTAYMELRSLRSDDTAVYYCARGGLREYYYAMDYWGQGTMVTVSS

SEQ ID NO: 31 - DNA, 363 bp, Artificial
  Recombinant DNA
  CDS (1)..(363)
caagtccagctggtgcagtctggggctgaagtgaagaagcctggggcctcagtgaaagtctcctgcaagggttccggctacacattcactgattatgctatgcactgggtgcgacaggcccctggacaaggcctggagtggattggagttattagtacttactatggtaatacaaactacaaccagaagtttaagggcaaggccacaatgactgtcgacacatccaccagcacagcctatatggaacttaggagcttgagatctgacgatactgccgtgtattactgtgcaagaggaggattgcgagagtattactatgctatggactactggggtcaaggaaccatggtcaccgtctcctca

SEQ ID NO: 32 - protein, 121 aa, Artificial
  Synthetic Construct (Recombinant Protein)
QVQLVQSGAEVKKPGASVKVSCKGSGYTFTDYAMHWVRQAPGQGLEWIGVISTYYGNTNYNQKFKGKATMTVDTSTSTAYMELRSLRSDDTAVYYCARGGLREYYYAMDYWGQGTMVTVSS

SEQ ID NO: 33 - DNA, 363 bp, Artificial
  Recombinant DNA
  CDS (1)..(363)
caagtccagctggtgcagtctggggctgaagtgaagaagcctggggcctcagtgaaagtctcctgcaaggcttccggctacacattcactgattatgctatgcactgggtgcgacaggcccctggacaaggcctggagtggattggagttattagtacttactatggtaatacaaactacaaccagaagtttaagggcaaggccacaatgactgtcgacaaatccaccagcacagcctatatggaacttaggagcttgagatctgacgatactgccgtgtattactgtgcaagaggaggattgcgagagtattactatgctatggactactggggtcaaggaaccatggtcaccgtctcctca

SEQ ID NO: 34 - protein, 121 aa, Artificial
  Synthetic Construct (Recombinant Protein)
QVQLVQSGAEVKKPGASVKVSCKASGYTFTDYAMHWVRQAPGQGLEWIGVISTYYGNTNYNQKFKGKATMTVDKSTSTAYMELRSLRSDDTAVYYCARGGLREYYYAMDYWGQGTMVTVSS

SEQ ID NO: 35 - DNA, 363 bp, Artificial
  Recombinant DNA
  CDS (1)..(363)
caagtccagctggtgcagtctggggctgaagtgaagaagcctggggcctcagtgaaagtctcctgcaagggttccggctacacattcactgattatgctatgcactgggtgcgacaggcccctggacaaggcctggagtggattggagttattagtacttactatggtaatacaaactacaaccagaagtttaagggcaaggccacaatgactgtcgacaaatccaccagcacagcctatatggaacttaggagcttgagatctgacgatactgccgtgtattactgtgcaagaggaggattgcgagagtattactatgctatggactactggggtcaaggaaccatggtcaccgtctcctca

SEQ ID NO: 36 - protein, 121 aa, Artificial
  Synthetic Construct (Recombinant Protein)
QVQLVQSGAEVKKPGASVKVSCKGSGYTFTDYAMHWVRQAPGQGLEWIGVISTYYGNTNYNQKFKGKATMTVDKSTSTAYMELRSLRSDDTAVYYCARGGLREYYYAMDYWGQGTMVTVSS

SEQ ID NO: 37 - DNA, 363 bp, Artificial
  Recombinant DNA
  CDS (1)..(363)
caagtccagctggtgcagtctggggctgaagtgaagaagcctggggcctcagtgaaagtctcctgcaaggcttccggctacacattcactgattatgctatgcactgggtgcgacaggcccctggacaaggcctggagtggattggagttattagtacttactatggtaatacaaactacaaccagaagtttaagggccgagccacaatgactgtcgacacatccaccagcacagcctatatggaacttaggagcttgagatctgacgatactgccgtgtattactgtgcaagaggaggattgcgagagtattactatgctatggactactggggtcaaggaaccatggtcaccgtctcctca

SEQ ID NO: 38 - protein, 121 aa, Artificial
  Synthetic Construct (Recombinant Protein)
QVQLVQSGAEVKKPGASVKVSCKASGYTFTDYAMHWVRQAPGQGLEWIGVISTYYGNTNYNQKFKGRATMTVDTSTSTAYMELRSLRSDDTAVYYCARGGLREYYYAMDYWGQGTMVTVSS

SEQ ID NO: 39 - DNA, 363 bp, Artificial
  Recombinant DNA
  CDS (1)..(363)
caagtccagctggtgcagtctggggctgaagtgaagaagcctggggcctcagtgaaagtctcctgcaagggttccggctacacattcactgattatgctatgcactgggtgcgacaggcccctggacaaggcctggagtggattggagttattagtacttactatggtaatacaaactacaaccagaagtttaagggccgagccacaatgactgtcgacacatccaccagcacagcctatatggaacttaggagcttgagatctgacgatactgccgtgtattactgtgcaagaggaggattgcgagagtattactatgctatggactactggggtcaaggaaccatggtcaccgtctcctca

SEQ ID NO: 40 - protein, 121 aa, Artificial
  Synthetic Construct (Recombinant Protein)
QVQLVQSGAEVKKPGASVKVSCKGSGYTFTDYAMHWVRQAPGQGLEWIGVISTYYGNTNYNQKFKGRATMTVDTSTSTAYMELRSLRSDDTAVYYCARGGLREYYYAMDYWGQGTMVTVSS

SEQ ID NO: 41 - DNA, 363 bp, Artificial
  Recombinant DNA
  CDS (1)..(363)
caagtccagctggtgcagtctggggctgaagtgaagaagcctggggcctcagtgaaagtctcctgcaaggcttccggctacacattcactgattatgctatgcactgggtgcgacaggcccctggacaaggcctggagtggattggagttattagtacttactatggtaatacaaactacaaccagaagtttaagggccgagccacaatgactgtcgacaaatccaccagcacagcctatatggaacttaggagcttgagatctgacgatactgccgtgtattactgtgcaagaggaggattgcgagagtattactatgctatggactactggggtcaaggaaccatggtcaccgtctcctca

SEQ ID NO: 42 - protein, 121 aa, Artificial
  Synthetic Construct (Recombinant Protein)
QVQLVQSGAEVKKPGASVKVSCKASGYTFTDYAMHWVRQAPGQGLEWIGVISTYYGNTNYNQKFKGRATMTVDKSTSTAYMELRSLRSDDTAVYYCARGGLREYYYAMDYWGQGTMVTVSS

SEQ ID NO: 43 - DNA, 363 bp, Artificial
  Recombinant DNA
  CDS (1)..(363)
caagtccagctggtgcagtctggggctgaagtgaagaagcctggggcctcagtgaaagtctcctgcaagggttccggctacacattcactgattatgctatgcactgggtgcgacaggcccctggacaaggcctggagtggattggagttattagtacttactatggtaatacaaactacaaccagaagtttaagggccgagccacaatgactgtcgacaaatccaccagcacagcctatatggaacttaggagcttgagatctgacgatactgccgtgtattactgtgcaagaggaggattgcgagagtattactatgctatggactactggggtcaaggaaccatggtcaccgtctcctca

SEQ ID NO: 44 - protein, 121 aa, Artificial
  Synthetic Construct (Recombinant Protein)
QVQLVQSGAEVKKPGASVKVSCKGSGYTFTDYAMHWVRQAPGQGLEWIGVISTYYGNTNYNQKFKGRATMTVDKSTSTAYMELRSLRSDDTAVYYCARGGLREYYYAMDYWGQGTMVTVSS

SEQ ID NO: 45 - DNA, 339 bp, Artificial
  Recombinant DNA
  CDS (1)..(339)
gacattgtcatgacacagtctccagactccctggctgtgtcactgggagagagggccactatcaactgcaagtccagtcagagccttctgaatagtagcaatcaaaagaactatttggcctggtaccagcagaaaccaggacagcctcctaaacttctggtctactttgcatccactagggaatctggggtccctgatcgcttcagtggcagtggatctgggacagatttcactcttaccatcagcagtctgcaggctgaagatgtggcagtttactactgtcagcaacattatagcactcctcccacattcggtcaggggaccaagctggagatcaaa

SEQ ID NO: 46 - protein, 113 aa, Artificial
  Synthetic Construct (Recombinant Protein)
DIVMTQSPDSLAVSLGERATINCKSSQSLLNSSNQKNYLAWYQQKPGQPPKLLVYFASTRESGVPDRFSGSGSGTDFTLTISSLQAEDVAVYYCQQHYSTPPTFGQGTKLEIK